European Patent Specification EP 4 153 302 B1, published May 29, 2024. Title: Treatment for viral respiratory infections. Applicant: Nasser, Syed Muhammad Tahir. The sequence listing filed with the application follows.

SEQUENCE LISTING (9 sequences)

SEQ ID NO: 1 - protein, 164 aa, Homo sapiens
TPVSQTTTAATASVRSTKDPCPSQPPVFPAAKQCPALEVTWPEVEVPLNGTLSLSCVACSRFPNFSILYWLGNGSFIEHLPGRLWEGSTSRERGSTGTQLCKALVLEQLTPALHSTNFSCVLVDPEQVVQRHVVLAQLWAGLRATLPPTQEALPSSHSSPQQQG

SEQ ID NO: 2 - protein, 85 aa, Homo sapiens
TPVSQTTTAATASVRSTKDPCPSQPPVFPAAKQCPALEVTWPEVEVPLSWAEGNLAPHPRSPALQPQQSTAAGLRLSTGPAAAQP

SEQ ID NO: 3 - protein, 168 aa, Homo sapiens
TPVSQTTTAATASVRSTKDPCPSQPPVFPAAKQCPALEVTWPEVEVPLNGTLSLSCVACSRFPNFSILYWLGNGSFIEHLPGRLWEGSTSRERGSTGTQLCKALVLEQLTPALHSTNFSCVLVDPEQVVQRHVVLAQLWVRSPRRGLQEQEELCFHMWGKGGLCQSSL

SEQ ID NO: 4 - protein, 132 aa, Homo sapiens
TPVSQTTTAATASVRSTKDPCPSQPPVFPAAKQCPALEVTWPEVEVPLNGTLSLSCVACSRFPNFSILYWLGNGSFIEHLPGRLWEGSTSRERGSTGWAEGNLAPHPRSPALQPQQSTAAGRLSTGPAAAQP

SEQ ID NO: 5 - protein, 218 aa, Molluscum contagiosum virus
MARGGKSGPRPWPDLLSRVRIVIVLVALLFLYSRACELEISTQVGPNGTTLLTCLGCTNHTHVSLMYWIVNESFPEQLDSSLSEGSTHKHKFPNQSLTEISTNLTVGPDVATHSTNFSCVLVDPEQVVQRHLVLTPPGTTPPTATPTATRTPPENADAAGARRRRRGAPKVVGTPPPKGNKKNKKNKKKGKGNKRRGNKTKHKNDKKRGGIPKNRHVR

SEQ ID NO: 6 - protein, 126 aa, Vaccinia virus
MRILFLIAFMYGCVHSYVNAVETKCPNLDIVTSSGEFHCSGCVEHMPEFSYMYWLAKDMKSDEDTKFIEHLGDGIKEDETVRTTDSGIVTLQKVLHVTDTNKFAHYRFTCVLATLDGVSKKNIWLK

SEQ ID NO: 7 - protein, 126 aa, Ectromelia virus
MRILFLIAFMYGCVHSYVNAVETKCPNLDIVTSSGEFHCSGCVEHMPEFSYMYWLAKDMKSDEDTKFIEHLGDGINEDETVRTTDGGITTLRKVLHVTDTNKFAHYRFTCVLTTLDGVSKKNIWLK

SEQ ID NO: 8 - protein, 161 aa, lumpy skin disease virus
MISFKKVVICLTLFTTFYVVYSKCAKKRDLVIYFPHKEGENVLLQCKGYSHHSNYAYVYWLIGNNNSFVEFMNGDIYKERMYFNKKPLKCGKEPRSDLIIKNVTEEIKNTNLTCVLMDLEEPIKKTLILNDIWNCLNNTCEHKNGISEKKVSESESKNVIE

SEQ ID NO: 9 - protein, 126 aa, Cowpox virus
MRILFLIAFMYGCVHSYVNAVETKCPNLDIVTSSGEFHCSGCVEHMPEFSYMYWLAKDMKSDEDTKFIEHLGDGIKEDETVRTTDGGITTLRKVLHVTDTNKFAHYRFTCVLTTLDGVSKKNIWLK